European Patent Specification EP 3 677 673 B1, published January 22, 2025. Title: A Glutamate Dehydrogenase Mutant and Its Application in Preparation of L-phosphinothricin. Applicant: ZHEJIANG UNIVERSITY. The sequence listing filed with the application follows.

SEQUENCE LISTING (22 sequences)

SEQ ID NO: 1 - protein, 449 aa, Artificial sequence
MSTMIESVDNFLARLKQRDPGQPEFHQAVEEVLRTLWPFLEANPHYLQSGILERMVEPERAVLFRVSWVDDQGKVQVNRGYRIQMSSAIGPYKGGLRFHPSVNLSVLKFLAFEQVFKNSLTSLPMGGGKGGSDFDPKGKSDAEVMRFCQAFMSELYRHIGADCDVPGGDIGVGAREIGFMFGQYKRLANQFTSVLTGKGMTYGGSLIRPEATGYGCVYFAEEMLKRQDKRIDGRRVAVSGSGNVAQYAARKVMDLGGKVISLSDSEGTLYAEAGLTDAQWDALMELKNVKRGRISELAGQFGLEFRKGQTPWSLPCDIALPCATQNELGAEDARTLLRNGCICVAEGANMPTTLEAVDIFLDAGILYAPGKASNAGGVAVSGLEMSQNAMRLLWTAGEVDSKLHNIMQSIHHACVHYGEEADGRINYVKGANIAGFVKVADAMLAQGVV

SEQ ID NO: 2 - protein, 449 aa, Artificial sequence
MSTMIESVDNFLARLKQRDPGQPEFHQAVEEVLRTLWPFLEANPHYLQSGILERMVEPERAVLFRVSWVDDQGKVQVNRGYRIQMSSAIGPYKGGLRFHPSVNLSVLKFLAFEQVFKNSLTSLPMGGGKGGSDFDPKGKSDAEVMRFCQAFMSELYRHIGADCDVPAGDIGVGAREIGFMFGQYKRLANQFTSVLTGKGMTYGGSLIRPEATGYGCVYFAEEMLKRQDKRIDGRRVAVSGSGNVAQYAARKVMDLGGKVISLSDSEGTLYAEAGLTDAQWDALMELKNVKRGRISELAGQFGLEFRKGQTPWSLPCDIALPCATQNELGAEDARTLLRNGCICVAEGANMPTTLEAVDIFLDAGILYAPGKASNAGGAAVSGLEMSQNAMRLLWTAGEVDSKLHNIMQSIHHACVHYGEEADGRINYVKGANIAGFVKVADAMLAQGVV

SEQ ID NO: 3 - protein, 447 aa, Artificial sequence
MTVDEQVSNYYDMLLKRNAGEPEFHQAVAEVLESLKIVLEKDPHYADYGLIQRLCEPERQLIFRVPWVDDQGQVHVNRGFRVQFNSALGPYKGGLRFHPSVNLGIVKFLGFEQIFKNSLTGLPIGGGKGGSDFDPKGKSDLEIMRFCQSFMTELHRHIGEYRDVPGGDIGVGGREIGYLFGHYRRMANQHESGVLTGKGLTWGGSLVRTEATGYGCVYFVSEMIKAKGESISGQKIIVSGSGNVATYAIEKAQELGATVIGFSDSSGWVHTPNGVDVAKLREIKEVRRARVSVYADEVEGATYHTDGSIWDLKCDIALPCATQNELNGENAKTLADNGCRFVAEGANMPSTPEAVEVFRERDIRFGPGKAANAGGVATSALEMQQNASRDSWSFEYTDERLQVIMKNIFKTCAETAAEYGHENDYVVGANIAGFKKVADAMLAQGVI

SEQ ID NO: 4 - protein, 447 aa, Artificial sequence
MTVDEQVSNYYDMLLKRNAGEPEFHQAVAEVLESLKIVLEKDPHYADYGLIQRLCEPERQLIFRVPWVDDQGQVHVNRGFRVQFNSALGPYKGGLRFHPSVNLGIVKFLGFEQIFKNSLTGLPIGGGKGGSDFDPKGKSDLEIMRFCQSFMTELHRHIGEYRDVPAGDIGVGGREIGYLFGHYRRMANQHESGVLTGKGLTWGGSLVRTEATGYGCVYFVSEMIKAKGESISGQKIIVSGSGNVATYAIEKAQELGATVIGFSDSSGWVHTPNGVDVAKLREIKEVRRARVSVYADEVEGATYHTDGSIWDLKCDIALPCATQNELNGENAKTLADNGCRFVAEGANMPSTPEAVEVFRERDIRFGPGKAANAGGAATSALEMQQNASRDSWSFEYTDERLQVIMKNIFKTCAETAAEYGHENDYVVGANIAGFKKVADAMLAQGVI

SEQ ID NO: 5 - protein, 446 aa, Artificial sequence
MIESVDHFLARLQQRDPAQPEFHQAVEEVLRSLWPFLEQNPHYLEAGILERMVEPERAVLFRVSWVDDQGKVQVNRGYRIQMSSAIGPYKGGLRFHPSVNLGVLKFLAFEQVFKNSLTSLPMGGGKGGSDFDPKGKSDAEVMRFCQAFMSELYRHIGADLDVPGGDIGVGAREIGFLFGQYKRLANQFTSVLTGKGMTYGGSLIRPEATGYGCVYFAEEMLKRQEQRIDGRRVAISGSGNVAQYAARKVMDLGGKVISLSDSEGTLFCEAGLTDEQWDALMELKNVKRGRISELAGRFGLEFRKGQTPWSLACDIALPCATQNELNADDARTLLRNGCICVAEGANMPTTLDAVDIFIEAGILYAPGKASNAGGVAVSGLEMSQNAMRLLWTAGEVDSKLHHIMQSIHHVCVHYGEEADGRINYVKGANIAGFVKVADAMLAQGVV

SEQ ID NO: 6 - protein, 446 aa, Artificial sequence
MIESVDHFLARLQQRDPAQPEFHQAVEEVLRSLWPFLEQNPHYLEAGILERMVEPERAVLFRVSWVDDQGKVQVNRGYRIQMSSAIGPYKGGLRFHPSVNLGVLKFLAFEQVFKNSLTSLPMGGGKGGSDFDPKGKSDAEVMRFCQAFMSELYRHIGADLDVPAGDIGVGAREIGFLFGQYKRLANQFTSVLTGKGMTYGGSLIRPEATGYGCVYFAEEMLKRQEQRIDGRRVAISGSGNVAQYAARKVMDLGGKVISLSDSEGTLFCEAGLTDEQWDALMELKNVKRGRISELAGRFGLEFRKGQTPWSLACDIALPCATQNELNADDARTLLRNGCICVAEGANMPTTLDAVDIFIEAGILYAPGKASNAGGAAVSGLEMSQNAMRLLWTAGEVDSKLHHIMQSIHHVCVHYGEEADGRINYVKGANIAGFVKVADAMLAQGVV

SEQ ID NO: 7 - protein, 457 aa, Artificial sequence
MTITTVSNEQLAKEYVDGVFEQLKQQNCHQAEFLQAAEEIFISLVPVFVQHPEYIKANILSRIVEPDRIISFRVAWQDDHNQVQVNRGYRVQYSNVMGPYKGGLRFHPSVNESIIKFLGFEQIFKNALTGQPIGGGKGGSNFDPKGKSDSEIMRFCQAFMTELYRHIGPDVDVPGGDIGVGAREVGYLWGQYKRLTKASESGVLTGKTPGYGGSLARKEATGYGTVYFVNEMLKDVNDSFEGKTVVVSGSGNVSTYAIEKAQQYGAKVVACSDSSGYIYDPEGLDLDVIKEIKEVKGDRISTYVSYRPNATFTNGCTGIWTIPCDIALPCATQNEINGESARTLISNGVKAIGEGANMPSDLEAINEFLNAGVLFGPAKAANAGGVAVSALEMAQDSSRVFWSFEEVDAKLHQIMKDIYSDSKAAAEKYGFPGNLVMGANIAGFIKVADGMLTEGIY

SEQ ID NO: 8 - protein, 457 aa, Artificial sequence
MTITTVSNEQLAKEYVDGVFEQLKQQNCHQAEFLQAAEEIFISLVPVFVQHPEYIKANILSRIVEPDRIISFRVAWQDDHNQVQVNRGYRVQYSNVMGPYKGGLRFHPSVNESIIKFLGFEQIFKNALTGQPIGGGKGGSNFDPKGKSDSEIMRFCQAFMTELYRHIGPDVDVPAGDIGVGAREVGYLWGQYKRLTKASESGVLTGKTPGYGGSLARKEATGYGTVYFVNEMLKDVNDSFEGKTVVVSGSGNVSTYAIEKAQQYGAKVVACSDSSGYIYDPEGLDLDVIKEIKEVKGDRISTYVSYRPNATFTNGCTGIWTIPCDIALPCATQNEINGESARTLISNGVKAIGEGANMPSDLEAINEFLNAGVLFGPAKAANAGGAAVSALEMAQDSSRVFWSFEEVDAKLHQIMKDIYSDSKAAAEKYGFPGNLVMGANIAGFIKVADGMLTEGIY

SEQ ID NO: 9 - protein, 423 aa, Artificial sequence
MAADKHTEEKGQQDDVLASTQIVIHRALEKLGYPEEVYELLKEPIRVLTVRIPVRMDDGSVKIFTGYRAQHNDAVGPTKGGVRFHPDVTEREVKALSIWMSLKCGIVDLPYGGGKGGIVCDPRTMSFRELERLSRGYVRAISQIVGPTKDIPGPDVFTNSQIMAWMMDEYSRIREFDSPGFITGKPLVLGGSHGRETATAKGVTICIREAAKKRGLSLEGARVVVQGFGNAGSYLAKFLHDAGAKVVGISDVYGALYDPNGLDIDYLLERRDSFGTVTKLFKNTISNKELLELDCDILVPAAIENQITAENAPRIKASIVVEAANGPTTLEATEILTQRGILLVPDVLASAGGVTVSYFEWVQNNQGYYWTEEEVEQRLEKVMVKAFNNVYEMAQTRRVDMRLAAYMVGVRKMAEACRFRGWV

SEQ ID NO: 10 - protein, 423 aa, Artificial sequence
MAADKHTEEKGQQDDVLASTQIVIHRALEKLGYPEEVYELLKEPIRVLTVRIPVRMDDGSVKIFTGYRAQHNDAVGPTKGGVRFHPDVTEREVKALSIWMSLKCGIVDLPYGGGKGGIVCDPRTMSFRELERLSRGYVRAISQIVGPTKDIPAPDVFTNSQIMAWMMDEYSRIREFDSPGFITGKPLVLGGSHGRETATAKGVTICIREAAKKRGLSLEGARVVVQGFGNAGSYLAKFLHDAGAKVVGISDVYGALYDPNGLDIDYLLERRDSFGTVTKLFKNTISNKELLELDCDILVPAAIENQITAENAPRIKASIVVEAANGPTTLEATEILTQRGILLVPDVLASAGGATVSYFEWVQNNQGYYWTEEEVEQRLEKVMVKAFNNVYEMAQTRRVDMRLAAYMVGVRKMAEACRFRGWV

SEQ ID NO: 11 - protein, 424 aa, Artificial sequence
MSAKQVSKDEEKEALNLFLSTQTIIKEALRKLGYPGDMYELMKEPQRMLTVRIPVKMDNGSVKVFTGYRSQHNDAVGPTKGGVRFHPEVNEEEVKALSIWMTLKCGIANLPYGGGKGGIICDPRTMSFGELERLSRGYVRAISQIVGPTKDIPGPDVYTNSQIMAWMMDEYSRLREFDSPGFITGKPLVLGGSQGRETATAQGVTICIEEAVKKKGIKLQNARIIIQGFGNAGSFLAKFMHDAGAKVIGISDANGGLYNPDGLDIPYLLDKRDSFGMVTNLFTDVITNEELLEKDCDILVPAAISNQITAKNAHNIQASIVVEAANGPTTIDATKILNERGVLLVPDILASAGGVTVSYFEWVQNNQGYYWSEEEVAEKLRSVMVSSFETIYQTAATHKVDMRLAAYMTGIRKSAEASRFRGWV

SEQ ID NO: 12 - protein, 424 aa, Artificial sequence
MSAKQVSKDEEKEALNLFLSTQTIIKEALRKLGYPGDMYELMKEPQRMLTVRIPVKMDNGSVKVFTGYRSQHNDAVGPTKGGVRFHPEVNEEEVKALSIWMTLKCGIANLPYGGGKGGIICDPRTMSFGELERLSRGYVRAISQIVGPTKDIPAPDVYTNSQIMAWMMDEYSRLREFDSPGFITGKPLVLGGSQGRETATAQGVTICIEEAVKKKGIKLQNARIIIQGFGNAGSFLAKFMHDAGAKVIGISDANGGLYNPDGLDIPYLLDKRDSFGMVTNLFTDVITNEELLEKDCDILVPAAISNQITAKNAHNIQASIVVEAANGPTTIDATKILNERGVLLVPDILASAGGATVSYFEWVQNNQGYYWSEEEVAEKLRSVMVSSFETIYQTAATHKVDMRLAAYMTGIRKSAEASRFRGWV

SEQ ID NO: 13 - protein, 426 aa, Artificial sequence
MVADKMQDSKNSQEEKHDVLKSTQTVIHKALEKLGYPDEVYELLKEPLRMMTVKIPVRMDDGSVKIFTGHRAQHNDAVGPTKGGIRFHPNVTEKEVKALSIWMSLKCGIVDLPYGGGKGGIVCDPRNMSFGELERLSRGYVRAISQIVGPTKDIPGPDVFTNSQIMAWMMDEYSRIDEFNSPGFITGKPLVLGGSHGRETATAKGVTICIREAAKKRGIELQGARVVVQGFGNAGSFLAKFMHDAGAKIVGISDAYGALHDPNGLDIDYLLDRRDSFGTVTKLFNNTISNKELLELDCDILVPAAIENQITEENAHNIQASIVVEAANGPTTLEATRILSERGILLVPDVLASAGGVTVSYFEWVQNNQGYYWTEEEVEEKLEKVMVKSFNNIYETSTTRKVDMRLAAYMIGVRKMAEGSRFRGWI

SEQ ID NO: 14 - protein, 426 aa, Artificial sequence
MVADKMQDSKNSQEEKHDVLKSTQTVIHKALEKLGYPDEVYELLKEPLRMMTVKIPVRMDDGSVKIFTGHRAQHNDAVGPTKGGIRFHPNVTEKEVKALSIWMSLKCGIVDLPYGGGKGGIVCDPRNMSFGELERLSRGYVRAISQIVGPTKDIPAPDVFTNSQIMAWMMDEYSRIDEFNSPGFITGKPLVLGGSHGRETATAKGVTICIREAAKKRGIELQGARVVVQGFGNAGSFLAKFMHDAGAKIVGISDAYGALHDPNGLDIDYLLDRRDSFGTVTKLFNNTISNKELLELDCDILVPAAIENQITEENAHNIQASIVVEAANGPTTLEATRILSERGILLVPDVLASAGGATVSYFEWVQNNQGYYWTEEEVEEKLEKVMVKSFNNIYETSTTRKVDMRLAAYMIGVRKMAEGSRFRGWI

SEQ ID NO: 15 - protein, 414 aa, Artificial sequence
MSENLNLFTSTQDVIQDALNKLGYDEAMYELLKEPLRMLQVRIPVKMDDGTTKVFTGYRAQHNDAVGPTKGGVRFHPQVSEEEVKALSMWMTLKCGIVDLPYGGGKGGVICDPRQMSMGEIERLSRGYVRAVSQIVGPTKDIPGPDVFTNAQIMAWMMDEYSRMDEFNSPGFITGKPLVLGGSQGRDRATAQGVTIVIEEAAKKRGIDIKGARVVIQGFGNAGSFLAKFMHDLGAKVIGISDAYGALHDPEGLDIDYLLDRRDSFGTVTTLFENTISNKELLELDCDILVPAAIENQITADNAHNIKADIVVEAANGPTTAEATKILTERGILLVPDVLASAGGVTVSYFEWVQNNQGYYWTEEEVEERLYKKMVEAFDNVYTTATTRNINMRLAAYMVGVRRTAEASRFRGWV

SEQ ID NO: 16 - protein, 414 aa, Artificial sequence
MSENLNLFTSTQDVIQDALNKLGYDEAMYELLKEPLRMLQVRIPVKMDDGTTKVFTGYRAQHNDAVGPTKGGVRFHPQVSEEEVKALSMWMTLKCGIVDLPYGGGKGGVICDPRQMSMGEIERLSRGYVRAVSQIVGPTKDIPAPDVFTNAQIMAWMMDEYSRMDEFNSPGFITGKPLVLGGSQGRDRATAQGVTIVIEEAAKKRGIDIKGARVVIQGFGNAGSFLAKFMHDLGAKVIGISDAYGALHDPEGLDIDYLLDRRDSFGTVTTLFENTISNKELLELDCDILVPAAIENQITADNAHNIKADIVVEAANGPTTAEATKILTERGILLVPDVLASAGGATVSYFEWVQNNQGYYWTEEEVEERLYKKMVEAFDNVYTTATTRNINMRLAAYMVGVRRTAEASRFRGWV

SEQ ID NO: 17 - protein, 450 aa, Artificial sequence
MSKYVDRVIAEVEKKYADEPEFVQTVEEVLSSLGPVVDAHPEYEEVALLERMVIPERVIEFRVPWEDDNGKVHVNTGYRVQFNGAIGPYKGGLRFAPSVNLSIMKFLGFEQAFKDSLTTLPMGGAKGGSDFDPNGKSDREVMRFCQAFMTELYRHIGPDIDVPGGDLGVGAREIGYMYGQYRKIVGGFYNGVLTGKARSFGGSLVRPEATGYGSVYYVEAVMKHENDTLVGKTVALAGFGNVAWGAAKKLAELGAKAVTLSGPDGYIYDPEGITTEEKINYMLEMRASGRNKVQDYADKFGVQFFPGEKPWGQKVDIIMPCATQNDVDLEQAKKIVANNIKYYIEVANMPTTNEALRFLMQQPNMVVAPSKAVNAGGVLVSGFEMSQNSERLSWTAEEVDSKLHQVMTDIHDGSAAAAERYGLGYNLVAGANIVGFQKIADAMMAQGIAW

SEQ ID NO: 18 - protein, 450 aa, Artificial sequence
MSKYVDRVIAEVEKKYADEPEFVQTVEEVLSSLGPVVDAHPEYEEVALLERMVIPERVIEFRVPWEDDNGKVHVNTGYRVQFNGAIGPYKGGLRFAPSVNLSIMKFLGFEQAFKDSLTTLPMGGAKGGSDFDPNGKSDREVMRFCQAFMTELYRHIGPDIDVPAGDLGVGAREIGYMYGQYRKIVGGFYNGVLTGKARSFGGSLVRPEATGYGSVYYVEAVMKHENDTLVGKTVALAGFGNVAWGAAKKLAELGAKAVTLSGPDGYIYDPEGITTEEKINYMLEMRASGRNKVQDYADKFGVQFFPGEKPWGQKVDIIMPCATQNDVDLEQAKKIVANNIKYYIEVANMPTTNEALRFLMQQPNMVVAPSKAVNAGGALVSGFEMSQNSERLSWTAEEVDSKLHQVMTDIHDGSAAAAERYGLGYNLVAGANIVGFQKIADAMMAQGIAW

SEQ ID NO: 19 - protein, 425 aa, Artificial sequence
MVTENTQGKEQKQESMNLLQSTQTVIKEALEKLGYQESMYELLKEPLRVLTVRIPVRMDNGEVKVFTGYRAQHNDAVGPTKGGIRFHPDVTEDEVKALSIWMSLKAGIVDLPYGGGKGGIICDPREMSFRELERLSRGYVRAVSQIVGPTKDIPGPDVFTNSQIMAWMMDEYSRIREFDSPGFITGKPIALGGSHGRETATAKGVTICIREAAKRRGIDLKGARVVVQGFGNAGSYLSKFMHDAGAKVVGISDAYGALYDPNGLDIDYLLDRRDSFGTVTKLFTNTITNKELLELDCDILVPAAIENQITAANAHNIKAKIVVEAANGPTTLEATKILTERGILLVPDVLASAGGVTVSYFEWVQNNQGYYWSEEEVQEKLEKVMVKAFENVYSLAQTRRVDMRLAAYMVGVRKMAEASRFRGWV

SEQ ID NO: 20 - protein, 425 aa, Artificial sequence
MVTENTQGKEQKQESMNLLQSTQTVIKEALEKLGYQESMYELLKEPLRVLTVRIPVRMDNGEVKVFTGYRAQHNDAVGPTKGGIRFHPDVTEDEVKALSIWMSLKAGIVDLPYGGGKGGIICDPREMSFRELERLSRGYVRAVSQIVGPTKDIPAPDVFTNSQIMAWMMDEYSRIREFDSPGFITGKPIALGGSHGRETATAKGVTICIREAAKRRGIDLKGARVVVQGFGNAGSYLSKFMHDAGAKVVGISDAYGALYDPNGLDIDYLLDRRDSFGTVTKLFTNTITNKELLELDCDILVPAAIENQITAANAHNIKAKIVVEAANGPTTLEATKILTERGILLVPDVLASAGGATVSYFEWVQNNQGYYWSEEEVQEKLEKVMVKAFENVYSLAQTRRVDMRLAAYMVGVRKMAEASRFRGWV

SEQ ID NO: 21 - protein, 261 aa, Artificial sequence
MYPDLKGKVVAITGAASGLGKAMAIRFGKEQAKVVINYYSNKQDPNEVKEEVIKAGGEAVVVQGDVTKEEDVKNIVQTAIKEFGTLDIMINNAGLENPVPSHEMPLKDWDKVIGTNLTGAFLGSREAIKYFVENDIKGNVINMSSVHEVIPWPLFVHYAASKGGIKLMTRTLALEYAPKGIRVNNIGPGAINTPINAEKFADPKQKADVESMIPMGYIGEPEEIAAVAAWLASKEASYVTGITLFADGGMTLYPSFQAGRG

SEQ ID NO: 22 - protein, 449 aa, Artificial sequence
MSTMIESVDNFLARLKQRDPGQPEFHQAVEEVLRTLWPFLEANPHYLQSGILERMVEPERAVLFRVSWVDDQGKVQVNRGYRIQMSSAIGPYKGGLRFHPSVNLSVLKFLAFEQVFKNSLTSLPMGGGKGGSDFDPKGKSDAEVMRFCQAFMSELYRHIGADCDVPGGDIGVGAREIGFMFGQYKRLANQFTSVLTGKGMTYGGSLIRPEATGYGCVYFAEEMLKRQDKRIDGRRVAVSGSGNVAQYAARKVMDLGGKVISLSDSEGTLYAEAGLTDAQWDALMELKNVKRGRISELAGQFGLEFRKGQTPWSLPCDIALPCATQNELGAEDARTLLRNGCICVAEGANMPTTLEAVDIFLDAGILYAPGKASNAGGAAVSGLEMSQNAMRLLWTAGEVDSKLHNIMQSIHHACVHYGEEADGRINYVKGANIAGFVKVADAMLAQGVV